European Patent Specification EP 4 117 706 B1, published September 4, 2024. Title: Fetuin A for treatment of renal disorders. Applicant: Universitaet Bern. The sequence listing filed with the application follows.

SEQUENCE LISTING (4 sequences)

SEQ ID NO: 1 - protein, 368 aa, Human
MKSLVLLLCLAQLWGCHSAPHGPGLIYRQPNCDDPETEEAALVAIDYINQNLPWGYKHTLNQIDEVKVWPQQPSGELFEIEIDTLETTCHVLDPTPVARCSVRQLKEHAVEGDCDFQLLKLDGKFSVVYAKCDSSPADSAEDVRKVCQDCPLLAPLNDTRVVHAAKAALAAFNAQNNGSNFQLEEISRAQLVPLPPSTYVEFTVSGTDCVAKEATEAAKCNLLAEKQYGFCKATLSEKLGGAEVAVTCMVFQTQPVSSQPQPEGANEAVPTPVVDPDAPPSPPLGAPGLPPAGSPPDSHVLLAAPPGHQLHRAHYDLRHTFMGVVSLGSPSGEVSHPRKTRTVVQPSVGAAAGPVVPPCPGRIRHFKV

SEQ ID NO: 2 - DNA, 1107 bp, Human
atgaagtccctcgtcctgctcctttgtcttgctcagctctggggctgccactcagccccacatggcccagggctgatttatagacaaccgaactgcgatgatccagaaactgaggaagcagctctggtggctatagactacatcaatcaaaaccttccttggggatacaaacacaccttgaaccagattgatgaagtaaaggtgtggcctcagcagccctccggagagctgtttgagattgaaatagacaccctggaaaccacctgccatgtgctggaccccacccctgtggcaagatgcagcgtgaggcagctgaaggagcatgctgtcgaaggagactgtgatttccagctgttgaaactagatggcaagttttccgtggtatacgcaaaatgtgattccagtccagcagactcagccgaggacgtgcgcaaggtgtgccaagactgccccctgctggccccgctgaacgacaccagggtggtgcacgccgcgaaagctgccctggccgccttcaacgctcagaacaacggctccaattttcagctggaggaaatttcccgggctcagcttgtgcccctcccaccttctacctatgtggagtttacagtgtctggcactgactgtgttgctaaagaggccacagaggcagccaagtgtaacctgctggcagaaaagcaatatggcttttgtaaggcaacactcagtgagaagcttggtggggcagaggttgcagtgacctgcatggtgttccaaacacagcccgtgagctcacagccccaaccagaaggtgccaatgaagcagtccccacacccgtggtggacccagatgcacctccgtcccctccacttggcgcacctggactccctccagctggctcacccccagactcccatgtgttactggcagctcctccaggacaccagttgcaccgggcgcactacgacctgcgccacaccttcatgggtgtggtctcattggggtcaccctcaggagaagtgtcgcacccccggaaaacacgcacagtggtgcagcctagtgttggtgctgctgctgggccagtggttcctccatgtccggggaggatcagacacttcaaggtctag

SEQ ID NO: 3 - protein, 359 aa, Bovine
MKSFVLLFCLAQLWGCHSIPLDPVAGYKEPACDDPDTEQAALAAVDYINKHLPRGYKHTLNQIDSVKVWPRRPTGEVYDIEIDTLETTCHVLDPTPLANCSVRQQTQHAVEGDCDIHVLKQDGQFSVLFTKCDSSPDSAEDVRKLCPDCPLLAPLNDSRVVHAVEVALATFNAESNGSYLQLVEISRAQFVPLPVSVSVEFAVAATDCIAKEVVDPTKCNLLAEKQYGFCKGSVIQKALGGEDVRVTCTLFQTQPVIPQPQPDGAEAEAPSAVPDAAGPTPSAAGPPVASVVVGPSVVAVPLPLHRAHYDLRHTFSGVASVESSSGEAFHVGKTPIVGQPSIPGGPVRLCPGRIRYFKI

SEQ ID NO: 4 - DNA, 1080 bp, Bovine
atgaaatccttcgttctgctcttttgcctggctcagctctggggctgccactcgatcccgcttgacccggttgcaggttataaggaaccggcctgtgatgacccagacacagagcaagcagccttggctgccgtggactacatcaacaagcaccttcctcggggctacaagcacaccttgaaccagattgacagtgtgaaggtgtggccgaggcggcccacgggagaggtgtatgacattgaaatagataccctggaaaccacctgccacgtactggaccccacgcccctggcgaactgcagcgtgaggcagcagacgcagcacgcggtggaaggagactgcgatatccacgtgctgaaacaagatggccagttttccgtgctgtttacaaaatgtgattccagtccagattccgccgaggacgtgcgcaagttgtgcccagactgccccctgctggcgccactcaacgacagccgggtggtgcacgcagtggaggtcgcgctggctaccttcaatgccgagagcaacggctcctacttacagctggtggaaatttctcgggctcaatttgtgcctcttccagtttctgtctctgtggagtttgcagtggctgctactgactgtattgctaaagaagtcgtagatccaaccaagtgcaacctactggcagaaaagcaatatggcttctgtaaggggtcagtcattcagaaagctcttggtggggaggacgtcagagtgacttgcacgttgttccaaacgcagcctgtgattccgcagccccagcccgacggcgccgaggctgaggccccaagcgctgtgccggacgcagctgggcctacgccttctgcagctggcccgcccgtggcctccgtggtggtggggccaagcgtggtagcagttcccctgccgctgcaccgagcacactacgacttgcgccacactttctccggggtggcctcagtggagtcatcctcgggagaagcgttccacgtgggcaaaacacccatagtggggcagcctagcattcctggaggtccagtccgcctttgcccagggagaatcagatacttcaagatctag